European Patent Application EP 4 613 855 A1, published September 10, 2025. Title: MMLV REVERSE TRANSCRIPTASE MUTANT. Applicant: BGI SHENZHEN. Application CN. The sequence listing filed with the application follows.

SEQUENCE LISTING (12 sequences)

SEQ ID NO: 1 - DNA, 2016 bp, synthetic construct
  source 1..2016: mol_type = other DNA
atgctaaatatagaagatgagcatcggctacatgagacctcaaaagagccagatgtttctctagggtccacatggctgtctgattttcctcaggcctgggcggaaaccgggggcatgggactggcagttcgccaagctcctctgatcatacctctgaaagcaacctctacccccgtgtccataaaacaataccccatgtcacaagaagccagactggggatcaagccccacatacagagactgttggaccagggaatactggtaccctgccagtccccctggaacacgcccctgctacccgttaagaaaccagggactaatgattataggcctgtccaggatctgagagaagtcaacaagcgggtggaagacatccaccccaccgtgcccaacccttacaacctcttgagcgggctcccaccgtcccaccagtggtacactgtgcttgatttaaaggatgcctttttctgcctgagactccaccccaccagtcagcctctcttcgcctttgagtggagagatccagagatgggaatctcaggacaattgacctggaccagactcccacagggtttcaaaaacagtcccaccctgtttgatgaggcactgcacagagacctagcagacttccggatccagcacccagacttgatcctgctacagtacgtggatgacttactgctggccgccacttctgagctagactgccaacaaggtactcgggccctgttacaaaccctagggaacctcgggtatcgggcctcggccaagaaagcccaaatttgccagaaacaggtcaagtatctggggtatcttctaaaagagggtcagagatggctgactgaggccagaaaagagactgtgatggggcagcctactccgaagacccctcgacaactaagggagttcctagggacggcaggcttctgtcgcctctggatccctgggtttgcagaaatggcagcccccttgtaccctctcaccaaaacggggactctgtttaattggggcccagaccaacaaaaggcctatcaagaaatcaagcaagctcttctaactgccccagccctggggttgccagatttgactaagccctttgaactctttgtcgacgagaagcagggctacgccaaaggtgtcctaacgcaaaaactgggaccttggcgtcggccggtggcctacctgtccaaaaagctagacccagtagcagctgggtggcccccttgcctacggatggtagcagccattgccgtactgacaaaggatgcaggcaagctaaccatgggacagccactagtcattctggccccccatgcagtagaggcactagtcaaacaaccccccgaccgctggctttccaacgcccggatgactcactatcaggccttgcttttggacacggaccgggtccagttcggaccggtggtagccctgaacccggctacgctgctcccactgcctgaggaagggctgcaacacaactgccttgatatcctggccgaagcccacggaacccgacccgacctaacggaccagccgctcccagacgccgaccacacctggtacacggatggaagcagtctcttacaagagggacagcgtaaggcgggagctgcggtgaccaccgagaccgaggtaatctgggctaaagccctgccagccgggacatccgctcagcgggctgaactgatagcactcacccaggccctaaagatggcagaaggtaagaagctaaatgtttatactgatagccgttatgcttttgctactgcccatatccatggagaaatatacagaaggcgtgggttgctcacatcagaaggcaaagagatcaaaaataaagacgagatcttggccctactaaaagccctctttctgcccaaaagacttagcataatccattgtccaggacatcaaaagggacacagcgccgaggctagaggcaaccggatggctgaccaagcggcccgaaaggcagccatcacagagactccagacacctctaccctcctcata

SEQ ID NO: 2 - protein, 672 aa, synthetic construct
MLNIEDEHRLHETSKEPDVSLGSTWLSDFPQAWAETGGMGLAVRQAPLIIPLKATSTPVSIKQYPMSQEARLGIKPHIQRLLDQGILVPCQSPWNTPLLPVKKPGTNDYRPVQDLREVNKRVEDIHPTVPNPYNLLSGLPPSHQWYTVLDLKDAFFCLRLHPTSQPLFAFEWRDPEMGISGQLTWTRLPQGFKNSPTLFDEALHRDLADFRIQHPDLILLQYVDDLLLAATSELDCQQGTRALLQTLGNLGYRASAKKAQICQKQVKYLGYLLKEGQRWLTEARKETVMGQPTPKTPRQLREFLGTAGFCRLWIPGFAEMAAPLYPLTKTGTLFNWGPDQQKAYQEIKQALLTAPALGLPDLTKPFELFVDEKQGYAKGVLTQKLGPWRRPVAYLSKKLDPVAAGWPPCLRMVAAIAVLTKDAGKLTMGQPLVILAPHAVEALVKQPPDRWLSNARMTHYQALLLDTDRVQFGPVVALNPATLLPLPEEGLQHNCLDILAEAHGTRPDLTDQPLPDADHTWYTDGSSLLQEGQRKAGAAVTTETEVIWAKALPAGTSAQRAELIALTQALKMAEGKKLNVYTDSRYAFATAHIHGEIYRRRGLLTSEGKEIKNKDEILALLKALFLPKRLSIIHCPGHQKGHSAEARGNRMADQAARKAAITETPDTSTLLI

SEQ ID NO: 3 - DNA, 30 bp, synthetic construct
  source 1..30: mol_type = other DNA
aagcagtggtatcaacgcagagtacatggg

SEQ ID NO: 4 - DNA, 27 bp, synthetic construct
  source 1..27: mol_type = other DNA
gtgcttacttcttctttttgacctaca

SEQ ID NO: 5 - RNA, 203 nt, synthetic construct
  source 1..203: mol_type = other RNA
gggatgttggagtttagtgttattgaaagaggcgggtatattcctgcagtagaaaaaaataaggcattcctacgagcagatggttggaatgactattcctttgttacaatgttttatcttactgtctttgatgagcatggtgaaaaatgcgatatcggaaatgttaaaattggttttgtaggtcaaaaagaagaagtaagcac

SEQ ID NO: 6 - RNA, 70 nt, synthetic construct
  source 1..70: mol_type = other RNA
aatgatacggcgaccaccgagatctacactagatcgctcgtcggcagcgtcagatgtgtataagagacag

SEQ ID NO: 7 - DNA, 69 bp, synthetic construct
  source 1..69: mol_type = other DNA
tgtctcttatacacatctgacgctgccgacgagcgatctagtgtagatctcggtggtcgccgtatcatt

SEQ ID NO: 8 - DNA, 57 bp, synthetic construct
  source 1..57: mol_type = other DNA
aagcagtggtatcaacgcagagtacttttttttttttttttttttttttttttttvn

SEQ ID NO: 9 - DNA, 23 bp, synthetic construct
  source 1..23: mol_type = other DNA
aagcagtggtatcaacgcagagt

SEQ ID NO: 10 - DNA, 21 bp, synthetic construct
  source 1..21: mol_type = other DNA
atgataaatgtcgttagtttc

SEQ ID NO: 11 - DNA, 40 bp, synthetic construct
  source 1..40: mol_type = other DNA
ctgacgtcctgccaccggagaaactaacgacatttatcat

SEQ ID NO: 12 - DNA, 39 bp, synthetic construct
  source 1..39: mol_type = other DNA
cattagccagagcaaatatgctgacgtcctgccaccgga